European Patent Specification EP 3 333 261 B1, published November 15, 2023. Title: HEXURONATE C4-EPIMERASE VARIANTS WITH IMPROVED CONVERSION ACTIVITY TO D-TAGATOSE AND METHOD FOR PRODUCTION OF D-TAGATOSE USING THEM. Applicant: CJ CHEILJEDANG CORPORATION. The sequence listing filed with the application follows.

SEQUENCE LISTING (1 sequence)

SEQ ID NO: 1 - protein, 481 aa, A wild type of Hexuronate C4-epimerase
MVLKVFKDHFGRGYEVYEKSYREKDSLSFFLTKGEEGKILVVAGEKAPEGLSFFKKQRVEGVSFFFCERNHENLEVLRKYFPDLKPVRAGLRASFGTGDRLGITTPAHVRALKDSGLFPIFAQQSVRENERTGRTWRDVLDDATWGVFQEGYSEGFGADADHVKRPEDLVSAAREGFTMFTIDPSDHVRNLSKLSEREKNEMFEEILKKERIDRIYLGKKYTVLGERLEFDEKNLRDAALVYYDAIAHVDMMYQILKDETPDFDFEVSVDETETPTSPLFHIFVVEELRRRGVEFTNLALRFIGEWEKGIDYKGDLAQFEREIKMHAEIARMFEGYKISLHSGSDKFSVYPAFASATGGLFHVKTAGTSYLEAVKVISMVNPELFREIYRCALDHFEEDRKSYHISADLSKVPEVEKVKDEDLPGLFEDINVRQLIHVTYGSVLKDASLKERLFKTLEQNEELFYETVAKHIKRHVDLLKG